European Patent Application EP 4 257 608 A1, published October 11, 2023. Title: Antibody specific for CD47 and uses thereof. Applicant: InnoBation Bio Co., Ltd. The sequence listing filed with the application follows.

SEQUENCE LISTING (98 sequences)

SEQ ID NO: 1 - protein, 8 aa, Artificial Sequence
  7C7_VH_CDR1
GYTFTSYV

SEQ ID NO: 2 - protein, 8 aa, Artificial Sequence
  7C7_VH_CDR2
INPYNDGT

SEQ ID NO: 3 - protein, 13 aa, Artificial Sequence
  7C7_VH_CDR3
ARGRNRYDSWFAY

SEQ ID NO: 4 - protein, 6 aa, Artificial Sequence
  7C7_VL_CDR1
QDISNY

SEQ ID NO: 5 - protein, 3 aa, Artificial Sequence
  7C7_VL_CDR2
YTS

SEQ ID NO: 6 - protein, 9 aa, Artificial Sequence
  7C7_VL_CDR3
QQGNTLPWT

SEQ ID NO: 7 - protein, 120 aa, Artificial Sequence
  7C7_VH
EVQLQQSGPELVKPGASVRMSCKASGYTFTSYVMHWVKQKPGQGLEWIGYINPYNDGTKYNEKFKGKSTLTSDKSSSTAYMELSSLTSEDSAVYCCARGRNRYDSWFAYWGQGTLVTVSA

SEQ ID NO: 8 - protein, 107 aa, Artificial Sequence
  7C7_VL
DIQMTQTTSSLSASLGDRVTISCRASQDISNYLNWYQQKPDGTVKLLIYYTSRLHSGVPSRFSGSGSGTDYSLTISNLEQEDIATYFCQQGNTLPWTFGGGTKLEIK

SEQ ID NO: 9 - DNA, 360 bp, Artificial Sequence
  7C7_VH
gaggtccagctgcaacagtctggacctgagctggtaaagcctggggcctcagtgaggatgtcctgcaaggcttctggatacacattcactagctatgttatgcactgggtgaagcagaagcctgggcagggccttgagtggattggatatattaatccttacaatgatggtactaagtacaatgagaagttcaaaggcaagtccacactgacttcagacaaatcctccagcacagcctacatggagctcagcagcctgacctctgaggactctgcggtctattgctgtgcaagagggaggaataggtacgactcctggtttgcttactggggccaagggactctggtcactgtctctgca

SEQ ID NO: 10 - DNA, 321 bp, Artificial Sequence
  7C7_VL
gatatccagatgacacagactacatcctccctgtctgcctctctgggagacagagtcaccatcagttgcagggcaagtcaggacattagcaattatttaaactggtatcagcagaaaccagatggaactgttaaactcctgatctactacacatcaagattacactcaggagtcccatcaaggttcagtggcagtgggtctggaacagattactctctcaccattagcaacctggagcaagaagatattgccacttacttttgccaacagggtaatacgcttccgtggacgttcggtggaggcaccaagctggaaatcaaa

SEQ ID NO: 11 - protein, 8 aa, Artificial Sequence
  5H4_VH_CDR1
GYTFTNYW

SEQ ID NO: 12 - protein, 8 aa, Artificial Sequence
  5H4_VH_CDR2
IDPSDSYT

SEQ ID NO: 13 - protein, 10 aa, Artificial Sequence
  5H4_VH_CDR3
TRGGKRAMDY

SEQ ID NO: 14 - protein, 11 aa, Artificial Sequence
  5H4_VL_CDR1
QSLVHSNGNTY

SEQ ID NO: 15 - protein, 3 aa, Artificial Sequence
  5H4_VL_CDR2
KVS

SEQ ID NO: 16 - protein, 9 aa, Artificial Sequence
  5H4_VL_CDR3
SQSTHVPFT

SEQ ID NO: 17 - protein, 117 aa, Artificial Sequence
  5H4_VH
QVQLQQPGAELVKPGTSVKMSCKASGYTFTNYWMHWVKQRPGQVLEWIGVIDPSDSYTSYNQKFKGKATLTVDTSSTTAYMQLSSLTSEDSAVYYCTRGGKRAMDYWGQGTSVTVSS

SEQ ID NO: 18 - protein, 112 aa, Artificial Sequence
  5H4_VL
DVLMTQTPLSLPVSLGDQASISCRSSQSLVHSNGNTYLHWYLQKPGQSPKLLIYKVSNRFSGVPDRFSGSGSGTDFTLKISRVEAEDLGVYFCSQSTHVPFTFGSGTKLEIK

SEQ ID NO: 19 - DNA, 351 bp, Artificial Sequence
  5H4_VH
caggtccaactgcagcagcctggggctgagctggtgaagcctgggacttcagtgaagatgtcctgcaaggcttctggctacaccttcaccaactactggatgcactgggtgaagcagaggcctggacaagtccttgagtggatcggagtgattgatccttctgatagttatactagctacaatcaaaagttcaagggcaaggccacattgactgtagacacatcctccaccacagcctacatgcagctcagcagcctgacatctgaggactctgcggtctattactgtacaagagggggtaagagagctatggactactggggtcaaggaacctcagtcaccgtctcctca

SEQ ID NO: 20 - DNA, 336 bp, Artificial Sequence
  5H4_VL
gatgttttgatgacccaaactccactctccctgcctgtcagtcttggagatcaagcctccatctcttgcagatctagtcagagccttgtacacagtaatggaaacacctatttacattggtacctgcagaagccaggccagtctccaaagctcctgatctacaaagtttccaaccgattttctggggtcccagacaggttcagtggcagtggatcagggacagatttcacactcaagatcagcagagtggaggctgaggatctgggagtttatttctgctctcaaagtacacatgttccattcacgttcggctcggggacaaagttggaaataaaa

SEQ ID NO: 21 - protein, 8 aa, Artificial Sequence
  5A4_VH_CDR1
GYTFTNYW

SEQ ID NO: 22 - protein, 8 aa, Artificial Sequence
  5A4_VH_CDR2
IDPSNSAT

SEQ ID NO: 23 - protein, 9 aa, Artificial Sequence
  5A4_VH_CDR3
ARGGFAFDS

SEQ ID NO: 24 - protein, 11 aa, Artificial Sequence
  5A4_VL_CDR1
QSLVHSNGNTY

SEQ ID NO: 25 - protein, 3 aa, Artificial Sequence
  5A4_VL_CDR2
KVS

SEQ ID NO: 26 - protein, 9 aa, Artificial Sequence
  5A4_VL_CDR3
SQSTHVPWT

SEQ ID NO: 27 - protein, 116 aa, Artificial Sequence
  5A4_VH
QVQLQQPGPELVRPGASVKMSCKASGYTFTNYWIHWVKQRPGQGLEWIGMIDPSNSATRLNQKFKDKATLNVDKSSNTAYMQLSSLTSEDSAVYYCARGGFAFDSWGQGTTLTVSS

SEQ ID NO: 28 - protein, 112 aa, Artificial Sequence
  5A4_VL
DVLMTQTPLSLPVSLGDQASISCRSSQSLVHSNGNTYLHWYLQKPGQSPKLLIYKVSNRFSGVPDRFSGSGSGTDFTLKISRVEAEDLGVYFCSQSTHVPWTFGGGTKLEIK

SEQ ID NO: 29 - DNA, 348 bp, Artificial Sequence
  5A4_VH
caggtccaactgcagcagcctgggcctgagctggtgaggcctggggcttcagtgaagatgtcctgcaaggcttcaggctataccttcaccaactactggattcactgggtgaaacagaggcctggacaaggccttgagtggattggcatgattgatccttccaatagtgcaactaggttaaatcagaagttcaaggacaaggccacattgaatgtagacaaatcctccaacacagcctacatgcagctcagcagcctgacatctgaggactctgcagtctattactgtgcaagaggagggttcgcctttgactcctggggccaaggcaccactctcacagtctcctca

SEQ ID NO: 30 - DNA, 336 bp, Artificial Sequence
  5A4_VL
gatgttttgatgacccaaactccactctccctgcctgtcagtcttggagatcaagcctccatctcttgcagatctagtcagagccttgtacatagtaatggaaacacctatttacattggtacctgcagaagccaggccagtctccaaagctcctgatctacaaagtttccaaccgattttctggggtcccagacaggttcagtggcagtggatcagggacagatttcacactcaagatcagcagagtggaggctgaggatctgggagtttatttctgctctcaaagtacacatgttccgtggacgttcggtggaggcaccaagctggaaatcaaa

SEQ ID NO: 31 - protein, 8 aa, Artificial Sequence
  4E12_VH_CDR1
GYTFTNYG

SEQ ID NO: 32 - protein, 8 aa, Artificial Sequence
  4E12_VH_CDR2
INTYTGEP

SEQ ID NO: 33 - protein, 11 aa, Artificial Sequence
  4E12_VH_CDR3
ARGGGRGAMDY

SEQ ID NO: 34 - protein, 11 aa, Artificial Sequence
  4E12_VL_CDR1
QSIVHSNGNTY

SEQ ID NO: 35 - protein, 3 aa, Artificial Sequence
  4E12_VL_CDR2
KVS

SEQ ID NO: 36 - protein, 9 aa, Artificial Sequence
  4E12_VL_CDR3
FQGSHVPFT

SEQ ID NO: 37 - protein, 118 aa, Artificial Sequence
  4E12_VH
QIQFAQSGPELKKSGETVKISCRASGYTFTNYGMNWVKQAPGKGLKWMGWINTYTGEPTYADDFKGRFAFSLETSASTAYLQINNLKNEDMATYFCARGGGRGAMDYWGQGTTLTVSS

SEQ ID NO: 38 - protein, 112 aa, Artificial Sequence
  4E12_VL
DVLMTQTPLSLPVSLGDQASISCRSSQSIVHSNGNTYLDWYLQKPGQSPKLLIYKVSKRFSGVPDRFSGSGSGTDFTLKISRVEAEDLGVYYCFQGSHVPFTFGSGTKLEIK

SEQ ID NO: 39 - DNA, 354 bp, Artificial Sequence
  4E12_VH
cagatccagttcgcgcagtctggacctgagctgaagaagtctggagagacagtcaagatctcctgcagggcttctgggtataccttcacaaactatggaatgaactgggtgaagcaggctccaggaaagggtttaaagtggatgggctggataaacacctacactggagagccaacatatgctgatgacttcaagggacggtttgccttctctttggaaacctctgccagcactgcctatttgcagatcaacaacctcaaaaatgaggacatggctacatatttctgtgcaagagggggtgggaggggtgctatggactactggggccaaggcaccactctcacagtctcctca

SEQ ID NO: 40 - DNA, 336 bp, Artificial Sequence
  4E12_VL
gatgttttgatgacccaaactccactctccctgcctgtcagtcttggagatcaagcctccatctcttgcagatctagtcagagcattgtacatagtaatggaaacacctatttagactggtacctgcagaaaccaggccagtctccaaagctcctgatctacaaagtttccaaacgattttctggggtcccagacaggttcagtggcagtggatcagggacagatttcacactcaagatcagcagagtggaggctgaggatctgggagtttattactgctttcaaggttcacatgttccattcacgttcggctcggggacaaagttggaaataaaa

SEQ ID NO: 41 - protein, 8 aa, Artificial Sequence
  3H3_VH_CDR1
GYTFTNYW

SEQ ID NO: 42 - protein, 8 aa, Artificial Sequence
  3H3_VH_CDR2
IDPSNSET

SEQ ID NO: 43 - protein, 9 aa, Artificial Sequence
  3H3_VH_CDR3
ARGGFAFDS

SEQ ID NO: 44 - protein, 11 aa, Artificial Sequence
  3H3_VL_CDR1
QSLVHNNGNTY

SEQ ID NO: 45 - protein, 3 aa, Artificial Sequence
  3H3_VL_CDR2
KVS

SEQ ID NO: 46 - protein, 9 aa, Artificial Sequence
  3H3_VL_CDR3
SQSTHVPWT

SEQ ID NO: 47 - protein, 116 aa, Artificial Sequence
  3H3_VH
EVQLQQPGPELVRPGASVKMSCKASGYTFTNYWMHWVKQRPGQGLEWIGMIDPSNSETRLNQKFKDKATLNVDKSSNTAYMQLSSLTSEDSAVYSCARGGFAFDSWGQGTTLTVSS

SEQ ID NO: 48 - protein, 112 aa, Artificial Sequence
  3H3_VL
DVLMTQTPLSLPVSLGDQASISCRSSQSLVHNNGNTYLHWYLQKPGQSPKLLIYKVSNRFSGVPDRFRGSGSGTDFTLKISRVEAEDLGVYFCSQSTHVPWTFGGGTKLEIK

SEQ ID NO: 49 - DNA, 348 bp, Artificial Sequence
  3H3_VH
gaggtccagctgcagcagcctgggcctgagctggtgaggcctggggcttcagtgaagatgtcctgcaaggcttcaggctataccttcaccaactactggatgcactgggtgaaacagaggcctggacaaggccttgagtggattggcatgattgatccttccaatagtgaaactaggttaaatcagaagttcaaggacaaggccacattgaatgtagacaaatcctccaacacagcctacatgcagctcagcagcctgacatctgaggactctgcagtctattcctgtgcaagaggagggttcgcctttgactcctggggccaaggcaccactctcacagtctcctca

SEQ ID NO: 50 - DNA, 336 bp, Artificial Sequence
  3H3_VL
gatgttttgatgacccaaactccactctccctgcctgtcagtcttggagatcaagcctccatctcttgcagatctagtcagagccttgtacacaataatggaaacacctatttacattggtacctgcagaagccaggccagtctccaaagctcctgatctacaaagtttccaaccgattttctggggtcccagacaggttccgtggcagtggatcggggacagatttcacactcaagatcagcagagtggaggctgaggatctgggagtttatttctgctctcaaagtacacatgttccgtggacgttcggtggaggcaccaagctggaaatcaaa

SEQ ID NO: 51 - protein, 8 aa, Artificial Sequence
  3A5_VH_CDR1
GYTFTSYW

SEQ ID NO: 52 - protein, 8 aa, Artificial Sequence
  3A5_VH_CDR2
IDPSDSYT

SEQ ID NO: 53 - protein, 10 aa, Artificial Sequence
  3A5_VH_CDR3
ARGGKRAMDY

SEQ ID NO: 54 - protein, 11 aa, Artificial Sequence
  3A5_VL_CDR1
QSLVHSNGNTY

SEQ ID NO: 55 - protein, 3 aa, Artificial Sequence
  3A5_VL_CDR2
KVS

SEQ ID NO: 56 - protein, 9 aa, Artificial Sequence
  3A5_VL_CDR3
SQSTHVPFT

SEQ ID NO: 57 - protein, 117 aa, Artificial Sequence
  3A5_VH
EVQLQQPGAELVKPGASVKMSCKASGYTFTSYWMHWMNQRPGQGLEWIGVIDPSDSYTSYNQKFKGKATLTVDTSSSTAYMQLSSLTSEDSAVYYCARGGKRAMDYWGQGTSVTVSS

SEQ ID NO: 58 - protein, 112 aa, Artificial Sequence; identical to SEQ ID NO: 18
  3A5_VL

SEQ ID NO: 59 - DNA, 351 bp, Artificial Sequence
  3A5_VH
gaggtccagctgcagcagcctggggctgagctggtgaagcctggggcttcagtgaagatgtcctgcaaggcttctggctacaccttcaccagctactggatgcactggatgaaccagaggcctggacaaggccttgagtggatcggagtgattgatccttctgatagttatactagctacaatcaaaagttcaagggcaaggccacattgactgtagacacatcctccagcacagcctacatgcagctcagcagcctgacatctgaggactctgcggtctattactgtgcaagagggggtaagagagctatggactactggggtcaaggaacctcagtcaccgtctcctca

SEQ ID NO: 60 - DNA, 336 bp, Artificial Sequence; identical to SEQ ID NO: 20
  3A5_VL

SEQ ID NO: 61 - protein, 8 aa, Artificial Sequence
  1E7_VH_CDR1
GYIFTSYV

SEQ ID NO: 62 - protein, 8 aa, Artificial Sequence
  1E7_VH_CDR2
INPYNDGT

SEQ ID NO: 63 - protein, 9 aa, Artificial Sequence
  1E7_VH_CDR3
ARGGFTTDY

SEQ ID NO: 64 - protein, 11 aa, Artificial Sequence
  1E7_VL_CDR1
QSLVHSNGNTY

SEQ ID NO: 65 - protein, 3 aa, Artificial Sequence
  1E7_VL_CDR2
KVS

SEQ ID NO: 66 - protein, 732 aa, Artificial Sequence
  5H4_VL-Linker-VH
AAAAAAAAAAAAAAAAAAAAAAAAAAAAAAAAAAAAAAAAAAAAAAAAAAAAAAAAAAAAAAAAAAAAAAAAAAAAAAAAAAAAAAAAAAAAAAAAAAAAAAAAAAAAAAAAAAAAAAAAAAAAAAAAAAAAAAAAAAAAAAAAAAAAAAAAAAAAAAAAAAAAAAAAAAAAAAAAAAAAAAAAAAAAAAAAAAAAAAAAAAAAAAAAAAAAAAAAAAAAAAAAAAAAAAAAAAAAAAAAAAAAAAAAAAAAAAAAAAAAAAAAAAAAAAAAAAAAAAAAAAAAAAAAAAAAAAAAAAAAAAAAAAAAAAAAAAAAAAAAAAAAAAAAAAAAAAAAAAAAAAAAAAAAAAAAAAAAAAAAAAAAAAAAAAAAAAAAAAAAAAAAAAAAAAAAAAAAAAAAAAAAAAAAAAAAAAAAAAAAAAAAAAAAAAAAAAAAAAAAAAAAAAAAAAAAAAAAAAAAAAAAAAAAAAAAAAAAAAAAAAAAAAAAAAAAAAAAAAAAAAAAAAAAAAAAAAAAAAAAAAAAAAAAAAAAAAAAAAAAAAAAAAAAAAAAAAAAAAAAAAAAAAAAAAAAAAAAAAAAAAAAAAAAAAAAAAAAAAAAAAAAAAAAAAAAAAAAAAAAAAAAAAAAAAAAAAAAAAAAAAAAAAAAAAAAAAAAAAAAAAAAAAAAAAAAAAAAAAAAAAAAAAAAAAAAAAAAAAAAAAAAAAAAAAAAAAAAAAAAAAAAAAAAAAAA

SEQ ID NO: 67 - protein, 116 aa, Artificial Sequence
  1E7_VH
EVQLQQSGPELIKPGASVKMSCKASGYIFTSYVVYWVKQKPGQGLEWIGYINPYNDGTKYNEKFKGKATLTSYKSSSTAYMELSSLTSADSAVYYCARGGFTTDYWGQGTTLTVSS

SEQ ID NO: 68 - protein, 112 aa, Artificial Sequence
  1E7_VL
DVLMTQTPLSLPVSLGDQASISCRSSQSLVHSNGNTYLHWYLQKPGQSPKLLIYKVSNRFSGVPDRFSGSGSGTDFTLKISRVEAEDLGVYFCSQSTHVPYTFGGGTKLEIK

SEQ ID NO: 69 - DNA, 348 bp, Artificial Sequence
  1E7_VH
gaggtccagctgcaacagtctggacctgagctgataaagcctggggcttcagtgaagatgtcctgcaaggcttctggatacatattcactagttatgttgtgtattgggtgaagcagaagcctgggcagggccttgagtggattggatatattaatccttacaatgatggtactaagtacaatgagaagttcaagggcaaggccacactgacttcatacaaatcctccagcacagcctacatggagctcagcagcctgacctctgcggactctgcggtctattactgtgcaagaggggggtttactactgactactggggccaaggcaccactctcacagtctcctca

SEQ ID NO: 70 - DNA, 336 bp, Artificial Sequence
  1E7_VL
gatgttttgatgacccaaactccactctccctgcctgtcagtcttggagatcaagcctccatctcttgcagatctagtcagagccttgtacacagtaatggaaacacctatttacattggtacctgcagaagccaggccagtctccaaagctcctgatctacaaagtttccaaccgattttctggggtcccagacaggttcagtggcagtggatcagggacagatttcacactcaagatcagcagagtggaggctgaggatctgggagtttatttctgctctcaaagtacacatgttccttacacgttcggaggggggaccaagctggaaataaaa

SEQ ID NO: 71 - protein, 15 aa, Artificial Sequence
  Linker
GGGGSGGGGSGGGGS

SEQ ID NO: 72 - DNA, 45 bp, Artificial Sequence
  Linker
ggtggtggtggttcgggtggtggtggttcgggtggtggtggttcg

SEQ ID NO: 73 - protein, 242 aa, Artificial Sequence
  7C7_VL-Linker-VH
DIQMTQTTSSLSASLGDRVTISCRASQDISNYLNWYQQKPDGTVKLLIYYTSRLHSGVPSRFSGSGSGTDYSLTISNLEQEDIATYFCQQGNTLPWTFGGGTKLEIKGGGGSGGGGSGGGGSEVQLQQSGPELVKPGASVRMSCKASGYTFTSYVMHWVKQKPGQGLEWIGYINPYNDGTKYNEKFKGKSTLTSDKSSSTAYMELSSLTSEDSAVYCCARGRNRYDSWFAYWGQGTLVTVSA

SEQ ID NO: 74 - DNA, 726 bp, Artificial Sequence
  7C7_VL-Linker-VH
gatatccagatgacacagactacatcctccctgtctgcctctctgggagacagagtcaccatcagttgcagggcaagtcaggacattagcaattatttaaactggtatcagcagaaaccagatggaactgttaaactcctgatctactacacatcaagattacactcaggagtcccatcaaggttcagtggcagtgggtctggaacagattactctctcaccattagcaacctggagcaagaagatattgccacttacttttgccaacagggtaatacgcttccgtggacgttcggtggaggcaccaagctggaaatcaaaggtggtggtggttcgggtggtggtggttcgggtggtggtggttcggaggtccagctgcaacagtctggacctgagctggtaaagcctggggcctcagtgaggatgtcctgcaaggcttctggatacacattcactagctatgttatgcactgggtgaagcagaagcctgggcagggccttgagtggattggatatattaatccttacaatgatggtactaagtacaatgagaagttcaaaggcaagtccacactgacttcagacaaatcctccagcacagcctacatggagctcagcagcctgacctctgaggactctgcggtctattgctgtgcaagagggaggaataggtacgactcctggtttgcttactggggccaagggactctggtcactgtctctgca

SEQ ID NO: 75 - protein, 244 aa, Artificial Sequence
  5H4_VL-Linker-VH
DVLMTQTPLSLPVSLGDQASISCRSSQSLVHSNGNTYLHWYLQKPGQSPKLLIYKVSNRFSGVPDRFSGSGSGTDFTLKISRVEAEDLGVYFCSQSTHVPFTFGSGTKLEIKGGGGSGGGGSGGGGSQVQLQQPGAELVKPGTSVKMSCKASGYTFTNYWMHWVKQRPGQVLEWIGVIDPSDSYTSYNQKFKGKATLTVDTSSTTAYMQLSSLTSEDSAVYYCTRGGKRAMDYWGQGTSVTVSS

SEQ ID NO: 76 - DNA, 732 bp, Artificial Sequence
  5H4_VL-Linker-VH
gatgttttgatgacccaaactccactctccctgcctgtcagtcttggagatcaagcctccatctcttgcagatctagtcagagccttgtacacagtaatggaaacacctatttacattggtacctgcagaagccaggccagtctccaaagctcctgatctacaaagtttccaaccgattttctggggtcccagacaggttcagtggcagtggatcagggacagatttcacactcaagatcagcagagtggaggctgaggatctgggagtttatttctgctctcaaagtacacatgttccattcacgttcggctcggggacaaagttggaaataaaaggtggtggtggttcgggtggtggtggttcgggtggtggtggttcgcaggtccaactgcagcagcctggggctgagctggtgaagcctgggacttcagtgaagatgtcctgcaaggcttctggctacaccttcaccaactactggatgcactgggtgaagcagaggcctggacaagtccttgagtggatcggagtgattgatccttctgatagttatactagctacaatcaaaagttcaagggcaaggccacattgactgtagacacatcctccaccacagcctacatgcagctcagcagcctgacatctgaggactctgcggtctattactgtacaagagggggtaagagagctatggactactggggtcaaggaacctcagtcaccgtctcctca

SEQ ID NO: 77 - protein, 243 aa, Artificial Sequence
  5A4_VL-Linker-VH
DVLMTQTPLSLPVSLGDQASISCRSSQSLVHSNGNTYLHWYLQKPGQSPKLLIYKVSNRFSGVPDRFSGSGSGTDFTLKISRVEAEDLGVYFCSQSTHVPWTFGGGTKLEIKGGGGSGGGGSGGGGSQVQLQQPGPELVRPGASVKMSCKASGYTFTNYWIHWVKQRPGQGLEWIGMIDPSNSATRLNQKFKDKATLNVDKSSNTAYMQLSSLTSEDSAVYYCARGGFAFDSWGQGTTLTVSS

SEQ ID NO: 78 - DNA, 729 bp, Artificial Sequence
  5A4_VL-Linker-VH
gatgttttgatgacccaaactccactctccctgcctgtcagtcttggagatcaagcctccatctcttgcagatctagtcagagccttgtacatagtaatggaaacacctatttacattggtacctgcagaagccaggccagtctccaaagctcctgatctacaaagtttccaaccgattttctggggtcccagacaggttcagtggcagtggatcagggacagatttcacactcaagatcagcagagtggaggctgaggatctgggagtttatttctgctctcaaagtacacatgttccgtggacgttcggtggaggcaccaagctggaaatcaaaggtggtggtggttcgggtggtggtggttcgggtggtggtggttcgcaggtccaactgcagcagcctgggcctgagctggtgaggcctggggcttcagtgaagatgtcctgcaaggcttcaggctataccttcaccaactactggattcactgggtgaaacagaggcctggacaaggccttgagtggattggcatgattgatccttccaatagtgcaactaggttaaatcagaagttcaaggacaaggccacattgaatgtagacaaatcctccaacacagcctacatgcagctcagcagcctgacatctgaggactctgcagtctattactgtgcaagaggagggttcgcctttgactcctggggccaaggcaccactctcacagtctcctca

SEQ ID NO: 79 - protein, 245 aa, Artificial Sequence
  4E12_VL-Linker-VH
DVLMTQTPLSLPVSLGDQASISCRSSQSIVHSNGNTYLDWYLQKPGQSPKLLIYKVSKRFSGVPDRFSGSGSGTDFTLKISRVEAEDLGVYYCFQGSHVPFTFGSGTKLEIKGGGGSGGGGSGGGGSQIQFAQSGPELKKSGETVKISCRASGYTFTNYGMNWVKQAPGKGLKWMGWINTYTGEPTYADDFKGRFAFSLETSASTAYLQINNLKNEDMATYFCARGGGRGAMDYWGQGTTLTVSS

SEQ ID NO: 80 - DNA, 735 bp, Artificial Sequence
  4E12_VL-Linker-VH
gatgttttgatgacccaaactccactctccctgcctgtcagtcttggagatcaagcctccatctcttgcagatctagtcagagcattgtacatagtaatggaaacacctatttagactggtacctgcagaaaccaggccagtctccaaagctcctgatctacaaagtttccaaacgattttctggggtcccagacaggttcagtggcagtggatcagggacagatttcacactcaagatcagcagagtggaggctgaggatctgggagtttattactgctttcaaggttcacatgttccattcacgttcggctcggggacaaagttggaaataaaaggtggtggtggttcgggtggtggtggttcgggtggtggtggttcgcagatccagttcgcgcagtctggacctgagctgaagaagtctggagagacagtcaagatctcctgcagggcttctgggtataccttcacaaactatggaatgaactgggtgaagcaggctccaggaaagggtttaaagtggatgggctggataaacacctacactggagagccaacatatgctgatgacttcaagggacggtttgccttctctttggaaacctctgccagcactgcctatttgcagatcaacaacctcaaaaatgaggacatggctacatatttctgtgcaagagggggtgggaggggtgctatggactactggggccaaggcaccactctcacagtctcctca

SEQ ID NO: 81 - protein, 185 aa, Artificial Sequence
  3H3_VL-Linker-VH
RFSGVPDRFRGSGSGTDFTLKISRVEAEDLGVYFCSQSTHVPWTFGGGTKLEIKGGGGSGGGGSGGGGSEVQLQQPGPELVRPGASVKMSCKASGYTFTNYWMHWVKQRPGQGLEWIGMIDPSNSETRLNQKFKDKATLNVDKSSNTAYMQLSSLTSEDSAVYSCARGGFAFDSWGQGTTLTVSS

SEQ ID NO: 82 - DNA, 729 bp, Artificial Sequence
  3H3_VL-Linker-VH
gatgttttgatgacccaaactccactctccctgcctgtcagtcttggagatcaagcctccatctcttgcagatctagtcagagccttgtacacaataatggaaacacctatttacattggtacctgcagaagccaggccagtctccaaagctcctgatctacaaagtttccaaccgattttctggggtcccagacaggttccgtggcagtggatcggggacagatttcacactcaagatcagcagagtggaggctgaggatctgggagtttatttctgctctcaaagtacacatgttccgtggacgttcggtggaggcaccaagctggaaatcaaaggtggtggtggttcgggtggtggtggttcgggtggtggtggttcggaggtccagctgcagcagcctgggcctgagctggtgaggcctggggcttcagtgaagatgtcctgcaaggcttcaggctataccttcaccaactactggatgcactgggtgaaacagaggcctggacaaggccttgagtggattggcatgattgatccttccaatagtgaaactaggttaaatcagaagttcaaggacaaggccacattgaatgtagacaaatcctccaacacagcctacatgcagctcagcagcctgacatctgaggactctgcagtctattcctgtgcaagaggagggttcgcctttgactcctggggccaaggcaccactctcacagtctcctca

SEQ ID NO: 83 - protein, 244 aa, Artificial Sequence
  3A5_VL-Linker-VH
DVLMTQTPLSLPVSLGDQASISCRSSQSLVHSNGNTYLHWYLQKPGQSPKLLIYKVSNRFSGVPDRFSGSGSGTDFTLKISRVEAEDLGVYFCSQSTHVPFTFGSGTKLEIKGGGGSGGGGSGGGGSEVQLQQPGAELVKPGASVKMSCKASGYTFTSYWMHWMNQRPGQGLEWIGVIDPSDSYTSYNQKFKGKATLTVDTSSSTAYMQLSSLTSEDSAVYYCARGGKRAMDYWGQGTSVTVSS

SEQ ID NO: 84 - DNA, 732 bp, Artificial Sequence
  3A5_VL-Linker-VH
gatgttttgatgacccaaactccactctccctgcctgtcagtcttggagatcaagcctccatctcttgcagatctagtcagagccttgtacacagtaatggaaacacctatttacattggtacctgcagaagccaggccagtctccaaagctcctgatctacaaagtttccaaccgattttctggggtcccagacaggttcagtggcagtggatcagggacagatttcacactcaagatcagcagagtggaggctgaggatctgggagtttatttctgctctcaaagtacacatgttccattcacgttcggctcggggacaaagttggaaataaaaggtggtggtggttcgggtggtggtggttcgggtggtggtggttcggaggtccagctgcagcagcctggggctgagctggtgaagcctggggcttcagtgaagatgtcctgcaaggcttctggctacaccttcaccagctactggatgcactggatgaaccagaggcctggacaaggccttgagtggatcggagtgattgatccttctgatagttatactagctacaatcaaaagttcaagggcaaggccacattgactgtagacacatcctccagcacagcctacatgcagctcagcagcctgacatctgaggactctgcggtctattactgtgcaagagggggtaagagagctatggactactggggtcaaggaacctcagtcaccgtctcctca

SEQ ID NO: 85 - protein, 243 aa, Artificial Sequence
  1E7_VL-Linker-VH
DVLMTQTPLSLPVSLGDQASISCRSSQSLVHSNGNTYLHWYLQKPGQSPKLLIYKVSNRFSGVPDRFSGSGSGTDFTLKISRVEAEDLGVYFCSQSTHVPYTFGGGTKLEIKGGGGSGGGGSGGGGSEVQLQQSGPELIKPGASVKMSCKASGYIFTSYVVYWVKQKPGQGLEWIGYINPYNDGTKYNEKFKGKATLTSYKSSSTAYMELSSLTSADSAVYYCARGGFTTDYWGQGTTLTVSS

SEQ ID NO: 86 - DNA, 729 bp, Artificial Sequence
  1E7_VL-Linker-VH
gatgttttgatgacccaaactccactctccctgcctgtcagtcttggagatcaagcctccatctcttgcagatctagtcagagccttgtacacagtaatggaaacacctatttacattggtacctgcagaagccaggccagtctccaaagctcctgatctacaaagtttccaaccgattttctggggtcccagacaggttcagtggcagtggatcagggacagatttcacactcaagatcagcagagtggaggctgaggatctgggagtttatttctgctctcaaagtacacatgttccttacacgttcggaggggggaccaagctggaaataaaaggtggtggtggttcgggtggtggtggttcgggtggtggtggttcggaggtccagctgcaacagtctggacctgagctgataaagcctggggcttcagtgaagatgtcctgcaaggcttctggatacatattcactagttatgttgtgtattgggtgaagcagaagcctgggcagggccttgagtggattggatatattaatccttacaatgatggtactaagtacaatgagaagttcaagggcaaggccacactgacttcatacaaatcctccagcacagcctacatggagctcagcagcctgacctctgcggactctgcggtctattactgtgcaagaggggggtttactactgactactggggccaaggcaccactctcacagtctcctca

SEQ ID NO: 87 - DNA, 1178 bp, Artificial Sequence
  EF1 promoter
gctccggtgcccgtcagtgggcagagcgcacatcgcccacagtccccgagaagttggggggaggggtcggcaattgaaccggtgcctagagaaggtggcgcggggtaaactgggaaagtgatgtcgtgtactggctccgcctttttcccgagggtgggggagaaccgtatataagtgcagtagtcgccgtgaacgttctttttcgcaacgggtttgccgccagaacacaggtaagtgccgtgtgtggttcccgcgggcctggcctctttacgggttatggcccttgcgtgccttgaattacttccacctggctgcagtacgtgattcttgatcccgagcttcgggttggaagtgggtgggagagttcgaggccttgcgcttaaggagccccttcgcctcgtgcttgagttgaggcctggcctgggcgctggggccgccgcgtgcgaatctggtggcaccttcgcgcctgtctcgctgctttcgataagtctctagccatttaaaatttttgatgacctgctgcgacgctttttttctggcaagatagtcttgtaaatgcgggccaagatctgcacactggtatttcggtttttggggccgcgggcggcgacggggcccgtgcgtcccagcgcacatgttcggcgaggcggggcctgcgagcgcggccaccgagaatcggacgggggtagtctcaagctggccggcctgctctggtgcctggcctcgcgccgccgtgtatcgccccgccctgggcggcaaggctggcccggtcggcaccagttgcgtgagcggaaagatggccgcttcccggccctgctgcagggagctcaaaatggaggacgcggcgctcgggagagcgggcgggtgagtcacccacacaaaggaaaagggcctttccgtcctcagccgtcgcttcatgtgactccactgagtaccgggcgccgtccaggcacctcgattagttctcgagcttttggagtacgtcgtctttaggttggggggaggggttttatgcgatggagtttccccacactgagtgggtggagactgaagttaggccagcttggcacttgatgtaattctccttggaatttgccctttttgagtttggatcttggttcattctcaagcctcagacagtggttcaaagtttttttcttccatttcaggtgtcgtga

SEQ ID NO: 88 - DNA, 63 bp, Artificial Sequence
  signal peptide
atggccttaccagtgaccgccttgctcctgccgctggccttgctgctccacgccgccaggccg

SEQ ID NO: 89 - DNA, 135 bp, Artificial Sequence
  CD8 Hinge
accacgacgccagcgccgcgaccaccaacaccggcgcccaccatcgcgtcgcagcccctgtccctgcgcccagaggcgtgccggccagcggcggggggcgcagtgcacacgagggggctggacttcgcctgtgat

SEQ ID NO: 90 - DNA, 72 bp, Artificial Sequence
  transmembrane domain
atctacatctgggcgcccttggccgggacttgtggggtccttctcctgtcactggttatcaccctttactgc

SEQ ID NO: 91 - DNA, 126 bp, Artificial Sequence
  4-1BB
aaacggggcagaaagaaactcctgtatatattcaaacaaccatttatgagaccagtacaaactactcaagaggaagatggctgtagctgccgatttccagaagaagaagaaggaggatgtgaactg

SEQ ID NO: 92 - DNA, 336 bp, Artificial Sequence
  CD3zeta
agagtgaagttcagcaggagcgcagacgcccccgcgtacaagcagggccagaaccagctctataacgagctcaatctaggacgaagagaggagtacgatgttttggacaagagacgtggccgggaccctgagatggggggaaagccgagaaggaagaaccctcaggaaggcctgtacaatgaactgcagaaagataagatggcggaggcctacagtgagattgggatgaaaggcgagcgccggaggggcaaggggcacgatggcctttaccagggtctcagtacagccaccaaggacacctacgacgcccttcacatgcaggccctgccccctcgc

SEQ ID NO: 93 - DNA, 591 bp, Artificial Sequence
  WPRE
atcaacctctggattacaaaatttgtgaaagattgactggtattcttaactatgttgctccttttacgctatgtggatacgctgctttaatgcctttgtatcatgctattgcttcccgtatggctttcattttctcctccttgtataaatcctggttgctgtctctttatgaggagttgtggcccgttgtcaggcaacgtggcgtggtgtgcactgtgtttgctgacgcaacccccactggttggggcattgccaccacctgtcagctcctttccgggactttcgctttccccctccctattgccacggcggaactcatcgccgcctgccttgcccgctgctggacaggggctcggctgttgggcactgacaattccgtggtgttgtcggggaagctgacgtcctttccatggctgctcgcctgtgttgccacctggattctgcgcgggacgtccttctgctacgtcccttcggccctcaatccagcggaccttccttcccgcggcctgctgccggctctgcggcctcttccgcgtcttcgccttcgccctcagacgagtcggatctccctttgggccgcctccccgcctg

SEQ ID NO: 94 - protein, 21 aa, Artificial Sequence
  signal peptide
MALPVTALLLPLALLLHAARP

SEQ ID NO: 95 - protein, 45 aa, Artificial Sequence
  CD8 Hinge
TTTPAPRPPTPAPTIASQPLSLRPEACRPAAGGAVHTRGLDFACD

SEQ ID NO: 96 - protein, 24 aa, Artificial Sequence
  transmembrane domain
IYIWAPLAGTCGVLLLSLVITLYC

SEQ ID NO: 97 - protein, 42 aa, Artificial Sequence
  4-1BB
KRGRKKLLYIFKQPFMRPVQTTQEEDGCSCRFPEEEEGGCEL

SEQ ID NO: 98 - protein, 112 aa, Artificial Sequence
  CD3zeta
RVKFSRSADAPAYKQGQNQLYNELNLGRREEYDVLDKRRGRDPEMGGKPRRKNPQEGLYNELQKDKMAEAYSEIGMKGERRRGKGHDGLYQGLSTATKDTYDALHMQALPPR